European Patent Specification EP 3 240 572 B1, published November 1, 2023. Title: BENZAMIDE IMIDAZOPYRAZINE BTK INHIBITORS. Applicant: Merck Sharp & Dohme Corp. The sequence listing filed with the application follows.

SEQUENCE LISTING (1 sequence)

SEQ ID NO: 1 - protein, 15 aa, Artificial Sequence
  Completely Synthetic Amino Acid Sequence
EQEDEPEGDYFEWLE